European Patent Specification EP 4 125 376 B1, published July 15, 2026. Title: Antimicrobial Peptides. Applicant: Materias s.r.l. The sequence listing filed with the application follows.

SEQUENCE LISTING (33 sequences)

SEQ ID NO: 1 - protein, 10 aa, Artificial Sequence
  AMP
RLKWVRIWRR

SEQ ID NO: 2 - protein, 10 aa, Artificial Sequence
  AMP
KLRWVRIWRR

SEQ ID NO: 3 - protein, 10 aa, Artificial Sequence
  AMP
RLRWVRIWRR

SEQ ID NO: 4 - protein, 10 aa, Artificial Sequence
  AMP
KLKWVRIWRR

SEQ ID NO: 5 - protein, 10 aa, Artificial Sequence
  AMP
RLKWVKIWRR

SEQ ID NO: 6 - protein, 10 aa, Artificial Sequence
  AMP
KLRWVKIWRR

SEQ ID NO: 7 - protein, 10 aa, Artificial Sequence
  AMP
RLRWVKIWRR

SEQ ID NO: 8 - protein, 10 aa, Artificial Sequence
  AMP
KLKWVKIWRR

SEQ ID NO: 9 - protein, 10 aa, Artificial Sequence
  AMP
RLKWVRIWKR

SEQ ID NO: 10 - protein, 10 aa, Artificial Sequence
  AMP
KLRWVRIWKR

SEQ ID NO: 11 - protein, 10 aa, Artificial Sequence
  AMP
RLRWVRIWKR

SEQ ID NO: 12 - protein, 10 aa, Artificial Sequence
  AMP
KLKWVRIWKR

SEQ ID NO: 13 - protein, 10 aa, Artificial Sequence
  AMP
RLKWVKIWKR

SEQ ID NO: 14 - protein, 10 aa, Artificial Sequence
  AMP
KLRWVKIWKR

SEQ ID NO: 15 - protein, 10 aa, Artificial Sequence
  AMP
RLRWVKIWKR

SEQ ID NO: 16 - protein, 10 aa, Artificial Sequence
  AMP
KLKWVKIWKR

SEQ ID NO: 17 - protein, 10 aa, Artificial Sequence
  AMP
RLKWVRIWRK

SEQ ID NO: 18 - protein, 10 aa, Artificial Sequence
  AMP
KLRWVRIWRK

SEQ ID NO: 19 - protein, 10 aa, Artificial Sequence
  AMP
RLRWVRIWRK

SEQ ID NO: 20 - protein, 10 aa, Artificial Sequence
  AMP
KLKWVRIWRK

SEQ ID NO: 21 - protein, 10 aa, Artificial Sequence
  AMP
RLKWVKIWRK

SEQ ID NO: 22 - protein, 10 aa, Artificial Sequence
  AMP
KLRWVKIWRK

SEQ ID NO: 23 - protein, 10 aa, Artificial Sequence
  AMP
RLRWVKIWRK

SEQ ID NO: 24 - protein, 10 aa, Artificial Sequence
  AMP
KLKWVKIWRK

SEQ ID NO: 25 - protein, 10 aa, Artificial Sequence
  AMP
RLKWVRIWKK

SEQ ID NO: 26 - protein, 10 aa, Artificial Sequence
  AMP
KLRWVRIWKK

SEQ ID NO: 27 - protein, 10 aa, Artificial Sequence
  AMP
RLRWVRIWKK

SEQ ID NO: 28 - protein, 10 aa, Artificial Sequence
  AMP
KLKWVRIWKK

SEQ ID NO: 29 - protein, 10 aa, Artificial Sequence
  AMP
RLKWVKIWKK

SEQ ID NO: 30 - protein, 10 aa, Artificial Sequence
  AMP
KLRWVKIWKK

SEQ ID NO: 31 - protein, 10 aa, Artificial Sequence
  AMP
RLRWVKIWKK

SEQ ID NO: 32 - protein, 10 aa, Artificial Sequence
  AMP
KLKWVKIWKK

SEQ ID NO: 33 - protein, 10 aa, Artificial Sequence
  HE10
VRLIVRIWRR